European Patent Application EP 4 613 859 A1, published September 10, 2025. Title: TLR 신호 억제 펩타이드 및 이를 포함하는 염증성 질환의 예방 또는 치료용 조성물. Applicant: 한국과학기술연구원. Application KR. The sequence listing filed with the application follows.

SEQUENCE LISTING (23 sequences)

SEQ ID NO: 1 - protein, 32 aa, synthetic construct
RQIKIWFQNRRMKWKKWFYERLVSLILRDTKV

SEQ ID NO: 2 - protein, 32 aa, synthetic construct
RQIKIWFQNRRMKWKKAFLYTFLINLTHPTNF

SEQ ID NO: 3 - protein, 32 aa, synthetic construct
RQIKIWFQNRRMKWKKAFFWAQLKSVLGNPTM

SEQ ID NO: 4 - protein, 32 aa, synthetic construct
RQIKIWFQNRRMKWKKRNFVAYLFQALANKGI

SEQ ID NO: 5 - protein, 32 aa, synthetic construct
RQIKIWFQNRRMKWKKTFLGHLYNALVQAGIH

SEQ ID NO: 6 - protein, 32 aa, synthetic construct
RQIKIWFQNRRMKWKKLFFWESLKQLLRSDGR

SEQ ID NO: 7 - protein, 32 aa, synthetic construct
RQIKIWFQNRRMKWKKYAFTGHLHRYLVQRGV

SEQ ID NO: 8 - protein, 32 aa, synthetic construct
RQIKIWFQNRRMKWKKSSFREGLWRLLELSKK

SEQ ID NO: 9 - protein, 32 aa, synthetic construct
RQIKIWFQNRRMKWKKPNLRTKVLNYLMRTKT

SEQ ID NO: 10 - protein, 32 aa, synthetic construct
RQIKIWFQNRRMKWKKNQWRNALTAAANLSGW

SEQ ID NO: 11 - protein, 32 aa, synthetic construct
RQIKIWFQNRRMKWKKRGFLSHLRHHLQAKDH

SEQ ID NO: 12 - protein, 32 aa, synthetic construct
RQIKIWFQNRRMKWKKKEVEGWRDALTKVASL

SEQ ID NO: 13 - protein, 32 aa, synthetic construct
RQIKIWFQNRRMKWKKDPQDLDWFYERLVSLF

SEQ ID NO: 14 - protein, 32 aa, synthetic construct
RQIKIWFQNRRMKWKKLGYHWIDWEYFVGIED

SEQ ID NO: 15 - protein, 32 aa, synthetic construct
RQIKIWFQNRRMKWKKDWVWDYLLPNLEGPAG

SEQ ID NO: 16 - protein, 32 aa, synthetic construct
RQIKIWFQNRRMKWKKWALDELLQILHARELF

SEQ ID NO: 17 - protein, 32 aa, synthetic construct
RQIKIWFQNRRMKWKKDPQDLDWFYERLVSLL

SEQ ID NO: 18 - protein, 34 aa, synthetic construct
RQIKIWFQNRRMKWKKDHHLDLPRGKAIKPEILG

SEQ ID NO: 19 - protein, 32 aa, synthetic construct
RQIKIWFQNRRMKWKKYTALTNSGFHTFRDND

SEQ ID NO: 20 - protein, 32 aa, synthetic construct
RQIKIWFQNRRMKWKKLVAHEISKKMKIFATI

SEQ ID NO: 21 - protein, 32 aa, synthetic construct
RQIKIWFQNRRMKWKKEWIREQLRPALKERLP

SEQ ID NO: 22 - protein, 32 aa, synthetic construct
RQIKIWFQNRRMKWKKGGAASSTTGGSSAATT

SEQ ID NO: 23 - protein, 16 aa, synthetic construct
RQIKIWFQNRRMKWKK